European Patent Application EP 4 129 323 A1, published February 8, 2023. Title: A modified HLA-B57 with increased expression levels. Applicant: ImmunOs Therapeutics AG. The sequence listing filed with the application follows.

SEQUENCE LISTING (20 sequences)

SEQ ID NO: 1 - protein, 280 aa, Homo sapiens
GSHSMRYFYTAMSRPGRGEPRFIAVGYVDDTQFVRFDSDAASPRMAPRAPWIEQEGPEYWDGETRNMKASAQTYRENLRIALRYYNQSEAGSHIIQVMYGCDVGPDGRLLRGHDQSAYDGKDYIALNEDLSSWTAADTAAQITQRKWEAARVAEQLRAYLEGLCVEWLRRYLENGKETLQRADPPKTHVTHHPISDHEATLRCWALGFYPAEITLTWQRDGEDQTQDTELVETRPAGDRTFQKWAAVVVPSGEEQRYTCHVQHEGLPKPLTLRWEPSSQS

SEQ ID NO: 2 - protein, 280 aa, Artificial Sequence
  HLA-B57:01MT
GSHSMRYFYTAMSRPGRGEPRFIAVGYVDDTQFVRFDSDAASPRMEPRAPWIEQEGPEYWDGETRNMKASAQTYRENLRIALRYYNQSEAGSHIIQRMYGCDVGPDGRLLRGHDQSAYDGKDYIALNEDLSSWTAADTAAQITQRKWEAARVAEQLRAYLEGLCVEWLRRYLENGKETLQRADPPKTHVTHHPISDHEATLRCWALGFYPAEITLTWQRDGEDQTQDTELVETRPAGDRTFQKWAAVVVPSGEEQRYTCHVQHEGLPKPLTLRWEPSSQS

SEQ ID NO: 3 - protein, 10 aa, Artificial Sequence
  peptide linker
GGGGSGGGGS

SEQ ID NO: 4 - protein, 228 aa, Homo sapiens
ESKYGPPCPPCPAPEFLGGPSVFLFPPKPKDTLMISRTPEVTCVVVDVSQEDPEVQFNWYVDGVEVHNAKTKPREEQFNSTYRVVSVLTVLHQDWLNGKEYKCKVSNKGLPSSIEKTISKAKGQPREPQVYTLPPSQEEMTKNQVSLTCLVKGFYPSDIAVEWESNGQPENNYKTTPPVLDSDGSFFLYSRLTVDKSRWQEGNVFSCSVMHEALHNHYTQKSLSLSLG

SEQ ID NO: 5 - protein, 540 aa, Artificial Sequence
  Recombinant HLAB57 fusion protein amino acid
AAAMNFGLRLIFLVLTLKGVQCGSHSMRYFYTAMSRPGRGEPRFIAVGYVDDTQFVRFDSDAASPRMEPRAPWIEQEGPEYWDGETRNMKASAQTYRENLRIALRYYNQSEAGSHIIQRMYGCDVGPDGRLLRGHDQSAYDGKDYIALNEDLSSWTAADTAAQITQRKWEAARVAEQLRAYLEGLCVEWLRRYLENGKETLQRADPPKTHVTHHPISDHEATLRCWALGFYPAEITLTWQRDGEDQTQDTELVETRPAGDRTFQKWAAVVVPSGEEQRYTCHVQHEGLPKPLTLRWEPSSQSGGGGSGGGGSESKYGPPCPPCPAPEFLGGPSVFLFPPKPKDTLMISRTPEVTCVVVDVSQEDPEVQFNWYVDGVEVHNAKTKPREEQFNSTYRVVSVLTVLHQDWLNGKEYKCKVSNKGLPSSIEKTISKAKGQPREPQVYTLPPSQEEMTKNQVSLTCLVKGFYPSDIAVEWESNGQPENNYKTTPPVLDSDGSFFLYSRLTVDKSRWQEGNVFSCSVMHEALHNHYTQKSLSLSLG

SEQ ID NO: 6 - DNA, 1626 bp, Artificial Sequence
  HLAB57 mutant fusion protein DNA
gcggccgccatgaattttggactgaggctgattttcctggtgctgaccctgaaaggcgtccagtgtggatcccactctatgagatacttctacaccgcaatgtctcgtcctggtcgcggggaacctagatttattgctgtgggatatgttgatgatactcaatttgtgcgttttgactccgacgcagcctcaccacggatggagcctagagcaccctggatagaacaagaagggcctgaatactgggatggtgaaacgcgaaacatgaaagcatcagctcaaacctatcgggagaacctgcgtatcgcactgagatactacaaccaatctgaggctggaagtcacattatccaacgtatgtatggttgtgacgtcggtcccgacggtcgcctgctccgtggtcatgaccaatcggcctatgacggaaaggattacatcgccttaaacgaggacctgagctcgtggactgccgcagatactgccgctcaaattacccaacggaagtgggaagcggcgcgcgtcgccgaacaactgcgagcctacctggagggcctgtgcgtcgagtggttgagacgctacctggagaacgggaaagagacgctgcaaagggccgatccccccaagacccatgtcacacatcacccgatctcggatcacgaagcaactctgcgatgctgggctcttgggttctaccccgctgagattacactgacttggcaaagggacggcgaagatcaaacacaagacaccgaacttgtggagactaggccagctggagatagaaccttccaaaagtgggctgccgtcgtcgtccctagtggagaggaacaacgatatacttgccacgtccaacacgaaggtttgccaaagcccctcactcttcgctgggaacctagctcgcaatcaggaggcggaggctcgggaggcggaggcagcgaaagcaaatacggtccaccctgcccaccttgcccggcgcctgaatttctgggcggaccttccgtgtttctgttccccccgaagcccaaggacaccctgatgatctcccggacccccgaagtgacctgcgtggtggtggacgtgtcccaggaagaccccgaagtccaatttaattggtatgtcgacggcgtcgaggtgcataatgccaagaccaagcccagagaggaacagttcaactccacctaccgggtggtgtccgtgctgaccgtgctgcaccaggactggctgaacggcaaagagtacaagtgcaaggtgtccaacaagggcctgccctcgtcaattgaaaagaccatctccaaggccaagggccagccccgcgagccccaggtgtacaccctgccccctagccaggaagagatgaccaagaaccaggtgtccctgacctgtctggtgaaaggcttctacccctccgacattgccgtggaatgggagtccaacggccagcccgagaacaactacaagaccaccccccctgtgctggactccgacggctccttcttcctgtactctcggctgacagtggataagtcccggtggcaggaaggcaacgtgttctcctgcagcgtgatgcacgaggccctgcacaaccactatacccagaagtccctgtccctgagcctgggctgatga

SEQ ID NO: 7 - protein, 280 aa, Homo sapiens
GSHSMRYFHTSVSRPGRGEPRFITVGYVDDTLFVRFDSDAASPREEPRAPWIEQEGPEYWDRETQICKAKAQTDREDLRTLLRYYNQSEAGSHTLQNMYGCDVGPDGRLLRGYHQDAYDGKDYIALNEDLSSWTAADTAAQITQRKWEAARVAEQLRAYLEGECVEWLRRYLENGKETLQRADPPKTHVTHHPISDHEATLRCWALGFYPAEITLTWQRDGEDQTQDTELVETRPAGDRTFQKWAAVVVPSGEEQRYTCHVQHEGLPKPLTLRWEPSSQS

SEQ ID NO: 8 - protein, 280 aa, Homo sapiens
GSHSMRYFHTSVSRPGRGEPRFITVGYVDDTLFVRFDSDAASPREEPRAPWIEQEGPEYWDRETQICKAKAQTDRESLRTLLRYYNQSEAGSHTLQNMYGCDVGPDGRLLRGYDQYAYDGKDYIALNEDLSSWTAADTAAQITQRKWEAAREAEQLRAYLEGECVEWLRRYLENGKETLQRADPPKTHVTHHPISDHEATLRCWALGFYPGEITLTWQRDGEDQTQDTELVETRPAGDRTFQKWAAVVVPSGEEQRYTCHVQHEGLPKPLTLRWEPSSQS

SEQ ID NO: 9 - protein, 280 aa, Homo sapiens
GSHSMRYFYTAMSRPGRGEPRFIAVGYVDDTQFVRFDSDAASPRTEPRAPWIEQEGPEYWDGETRNMKASAQTYRENLRIALRYYNQSEAGSHIIQRMYGCDLGPDGRLLRGHDQSAYDGKDYIALNEDLSSWTAADTAAQITQRKWEAARVAEQLRAYLEGLCVEWLRRYLENGKETLQRADPPKTHVTHHPVSDHEATLRCWALGFYPAEITLTWQRDGEDQTQDTELVETRPAGDRTFQKWAAVVVPSGEEQRYTCHVQHEGLPKPLTLRWEPSSQS

SEQ ID NO: 10 - protein, 280 aa, Homo sapiens
CSHSMRYFYTAVSRPGRGEPRFIAVGYVDDTQFVQFDSDAASPRGEPRAPWVEQEGPEYWDRETQKYKRQAQTDRVSLRNLRGYYNQSEAGSHTLQRMYGCDLGPDGRLLRGYNQFAYDGKDYIALNEDLRSWTAADTAAQITQRKWEAARTAEQLRAYLEGTCVEWLRRYLENGKKTLQRAEHPKTHVTHHPVSDHEATLRCWALGFYPAEITLTWQRDGEDQTQDTELVETRPAGDGTFQKWAAVVVPSGEEQRYTCHVQHEGLPEPLTLRWGPSSQS

SEQ ID NO: 11 - protein, 280 aa, Homo sapiens
CSHSMRYFSTSVSRPGRGEPRFIAVGYVDDTQFVRFDSDAASPRGEPRAPWVEQEGPEYWDRETQKYKRQAQTDRVSLRNLRGYYNQSEAGSHTLQRMFGCDLGPDGRLLRGYDQSAYDGKDYIALNEDLRSWTAADTAAQITQRKWEAAREAEQRRAYLEGTCVEWLRRYLENGKETLQRAEHPKTHVTHHPVSDHEATLRCWALGFYPAEITLTWQWDGEDQTQDTELVETRPAGDGTFQKWAAVVVPSGEEQRYTCHVQHEGLPEPLTLRWEPSSQP

SEQ ID NO: 12 - DNA, 1626 bp, Artificial Sequence
  HLAB57 wildtype fusion protein DNA
gcggccgccatgaactttggcctgcggctgatcttcctggtgctgaccctgaagggcgtgcagtgcggatcccactccatgcggtacttctacaccgccatgtcccggcctggacggggagagcctagattcattgccgtgggctacgtggacgacacccagttcgtcagattcgactccgacgccgcctctcctcggatggctcctagagccccttggatcgagcaggaaggccccgagtactgggacggcgagacacggaacatgaaggcctccgcccagacctacagagagaacctgagaatcgccctgcggtactacaaccagtccgaggccggctcccacatcatccaagtgatgtacggctgcgacgtgggccccgatggcagactgctgagaggccacgatcagtccgcctacgacggcaaggactatatcgccctgaacgaggacctgtcctcctggaccgctgccgataccgccgctcagatcactcagcggaagtgggaggccgccagagtggctgaacagctgagagcctacctggaaggcctgtgcgtggaatggctgcggagatacctggaaaacggcaaagagacactgcagcgggccgacccccctaagacccacgtgacccaccaccctatctccgaccacgaggccaccctgagatgttgggccctgggcttttaccccgccgagatcaccctgacctggcagagagatggcgaggaccagacccaggacaccgagctggtggaaaccagacctgccggcgaccggaccttccagaaatgggctgctgtggtggtgccctccggcgaggaacagagatacacctgtcacgtgcagcacgagggcctgcccaagcccctgactctgagatgggagccttccagccaatcaggaggcggaggctcgggaggcggaggcagcgaaagcaaatacggtccaccctgcccaccttgcccggcgcctgaatttctgggcggaccttccgtgtttctgttccccccgaagcccaaggacaccctgatgatctcccggacccccgaagtgacctgcgtggtggtggacgtgtcccaggaagaccccgaagtccaatttaattggtatgtcgacggcgtcgaggtgcataatgccaagaccaagcccagagaggaacagttcaactccacctaccgggtggtgtccgtgctgaccgtgctgcaccaggactggctgaacggcaaagagtacaagtgcaaggtgtccaacaagggcctgccctcgtcaattgaaaagaccatctccaaggccaagggccagccccgcgagccccaggtgtacaccctgccccctagccaggaagagatgaccaagaaccaggtgtccctgacctgtctggtgaaaggcttctacccctccgacattgccgtggaatgggagtccaacggccagcccgagaacaactacaagaccaccccccctgtgctggactccgacggctccttcttcctgtactctcggctgacagtggataagtcccggtggcaggaaggcaacgtgttctcctgcagcgtgatgcacgaggccctgcacaaccactatacccagaagtccctgtccctgagcctgggctgatga

SEQ ID NO: 13 - DNA, 373 bp, Homo sapiens
gcggccgccatgtcccggagcgttgcgctggctgtgttggccctgctctctctctccgggctggaagcaattcaacgtacacccaagattcaggtctatagtcgccaccccgctgagaatggaaagtctaattttctgaactgctatgtgtccggctttcatccctccgatattgaggttgacttactcaagaacggagagcgcatagaaaaggttgaacactctgacctcagttttagcaaggactggagtttctacttactgtactacactgaattcacccctaccgaaaaggacgaatacgcttgtcgtgtgaatcacgttactctgtctcaacccaaaattgtcaagtgggatcgggatatgtgataag

SEQ ID NO: 14 - protein, 122 aa, Homo sapiens
AAAMSRSVALAVLALLSLSGLEAIQRTPKIQVYSRHPAENGKSNFLNCYVSGFHPSDIEVDLLKNGERIEKVEHSDLSFSKDWSFYLLYYTEFTPTEKDEYACRVNHVTLSQPKIVKWDRDM

SEQ ID NO: 15 - protein, 518 aa, Artificial Sequence
  Recombinant HLA-B57 fusion protein
GSHSMRYFYTAMSRPGRGEPRFIAVGYVDDTQFVRFDSDAASPRMEPRAPWIEQEGPEYWDGETRNMKASAQTYRENLRIALRYYNQSEAGSHIIQRMYGCDVGPDGRLLRGHDQSAYDGKDYIALNEDLSSWTAADTAAQITQRKWEAARVAEQLRAYLEGLCVEWLRRYLENGKETLQRADPPKTHVTHHPISDHEATLRCWALGFYPAEITLTWQRDGEDQTQDTELVETRPAGDRTFQKWAAVVVPSGEEQRYTCHVQHEGLPKPLTLRWEPSSQSGGGGSGGGGSESKYGPPCPPCPAPEFLGGPSVFLFPPKPKDTLMISRTPEVTCVVVDVSQEDPEVQFNWYVDGVEVHNAKTKPREEQFNSTYRVVSVLTVLHQDWLNGKEYKCKVSNKGLPSSIEKTISKAKGQPREPQVYTLPPSQEEMTKNQVSLTCLVKGFYPSDIAVEWESNGQPENNYKTTPPVLDSDGSFFLYSRLTVDKSRWQEGNVFSCSVMHEALHNHYTQKSLSLSLG

SEQ ID NO: 16 - DNA, 1506 bp, Artificial Sequence
  HLAB57 mutant fusion protein DNA
gaacctagatttattgctgtgggatatgttgatgatactcaatttgtgcgttttgactccgacgcagcctcaccacggatggagcctagagcaccctggatagaacaagaagggcctgaatactgggatggtgaaacgcgaaacatgaaagcatcagctcaaacctatcgggagaacctgcgtatcgcactgagatactacaaccaatctgaggctggaagtcacattatccaacgtatgtatggttgtgacgtcggtcccgacggtcgcctgctccgtggtcatgaccaatcggcctatgacggaaaggattacatcgccttaaacgaggacctgagctcgtggactgccgcagatactgccgctcaaattacccaacggaagtgggaagcggcgcgcgtcgccgaacaactgcgagcctacctggagggcctgtgcgtcgagtggttgagacgctacctggagaacgggaaagagacgctgcaaagggccgatccccccaagacccatgtcacacatcacccgatctcggatcacgaagcaactctgcgatgctgggctcttgggttctaccccgctgagattacactgacttggcaaagggacggcgaagatcaaacacaagacaccgaacttgtggagactaggccagctggagatagaaccttccaaaagtgggctgccgtcgtcgtccctagtggagaggaacaacgatatacttgccacgtccaacacgaaggtttgccaaagcccctcactcttcgctgggaacctagctcgcaatcaggaggcggaggctcgggaggcggaggcagcgaaagcaaatacggtccaccctgcccaccttgcccggcgcctgaatttctgggcggaccttccgtgtttctgttccccccgaagcccaaggacaccctgatgatctcccggacccccgaagtgacctgcgtggtggtggacgtgtcccaggaagaccccgaagtccaatttaattggtatgtcgacggcgtcgaggtgcataatgccaagaccaagcccagagaggaacagttcaactccacctaccgggtggtgtccgtgctgaccgtgctgcaccaggactggctgaacggcaaagagtacaagtgcaaggtgtccaacaagggcctgccctcgtcaattgaaaagaccatctccaaggccaagggccagccccgcgagccccaggtgtacaccctgccccctagccaggaagagatgaccaagaaccaggtgtccctgacctgtctggtgaaaggcttctacccctccgacattgccgtggaatgggagtccaacggccagcccgagaacaactacaagaccaccccccctgtgctggactccgacggctccttcttcctgtactctcggctgacagtggataagtcccggtggcaggaaggcaacgtgttctcctgcagcgtgatgcacgaggccctgcacaaccactatacccagaagtccctgtccctgagcctgggctgatga

SEQ ID NO: 17 - protein, 540 aa, Artificial Sequence
  HLAB57 fusion protein
AAAMNFGLRLIFLVLTLKGVQCGSHSMRYFYTAMSRPGRGEPRFIAVGYVDDTQFVRFDSDAASPRMAPRAPWIEQEGPEYWDGETRNMKASAQTYRENLRIALRYYNQSEAGSHIIQVMYGCDVGPDGRLLRGHDQSAYDGKDYIALNEDLSSWTAADTAAQITQRKWEAARVAEQLRAYLEGLCVEWLRRYLENGKETLQRADPPKTHVTHHPISDHEATLRCWALGFYPAEITLTWQRDGEDQTQDTELVETRPAGDRTFQKWAAVVVPSGEEQRYTCHVQHEGLPKPLTLRWEPSSQSGGGGSGGGGSESKYGPPCPPCPAPEFLGGPSVFLFPPKPKDTLMISRTPEVTCVVVDVSQEDPEVQFNWYVDGVEVHNAKTKPREEQFNSTYRVVSVLTVLHQDWLNGKEYKCKVSNKGLPSSIEKTISKAKGQPREPQVYTLPPSQEEMTKNQVSLTCLVKGFYPSDIAVEWESNGQPENNYKTTPPVLDSDGSFFLYSRLTVDKSRWQEGNVFSCSVMHEALHNHYTQKSLSLSLG

SEQ ID NO: 18 - protein, 518 aa, Artificial Sequence
  HLA-B57 fusion protein amino acid
GSHSMRYFYTAMSRPGRGEPRFIAVGYVDDTQFVRFDSDAASPRMAPRAPWIEQEGPEYWDGETRNMKASAQTYRENLRIALRYYNQSEAGSHIIQVMYGCDVGPDGRLLRGHDQSAYDGKDYIALNEDLSSWTAADTAAQITQRKWEAARVAEQLRAYLEGLCVEWLRRYLENGKETLQRADPPKTHVTHHPISDHEATLRCWALGFYPAEITLTWQRDGEDQTQDTELVETRPAGDRTFQKWAAVVVPSGEEQRYTCHVQHEGLPKPLTLRWEPSSQSGGGGSGGGGSESKYGPPCPPCPAPEFLGGPSVFLFPPKPKDTLMISRTPEVTCVVVDVSQEDPEVQFNWYVDGVEVHNAKTKPREEQFNSTYRVVSVLTVLHQDWLNGKEYKCKVSNKGLPSSIEKTISKAKGQPREPQVYTLPPSQEEMTKNQVSLTCLVKGFYPSDIAVEWESNGQPENNYKTTPPVLDSDGSFFLYSRLTVDKSRWQEGNVFSCSVMHEALHNHYTQKSLSLSLG

SEQ ID NO: 19 - protein, 22 aa, Artificial Sequence
  secretory signal
AAAMNFGLRLIFLVLTLKGVQC

SEQ ID NO: 20 - protein, 539 aa, Artificial Sequence
  Recombinant HLA-B57 fusion protein
MASPAQLLFLLLLWLPDGVHAGSHSMRYFYTAMSRPGRGEPRFIAVGYVDDTQFVRFDSDAASPRMEPRAPWIEQEGPEYWDGETRNMKASAQTYRENLRIALRYYNQSEAGSHIIQRMYGCDVGPDGRLLRGHDQSAYDGKDYIALNEDLSSWTAADTAAQITQRKWEAARVAEQLRAYLEGLCVEWLRRYLENGKETLQRADPPKTHVTHHPISDHEATLRCWALGFYPAEITLTWQRDGEDQTQDTELVETRPAGDRTFQKWAAVVVPSGEEQRYTCHVQHEGLPKPLTLRWEPSSQSGGGGSGGGGSESKYGPPCPPCPAPEFLGGPSVFLFPPKPKDTLMISRTPEVTCVVVDVSQEDPEVQFNWYVDGVEVHNAKTKPREEQFNSTYRVVSVLTVLHQDWLNGKEYKCKVSNKGLPSSIEKTISKAKGQPREPQVYTLPPSQEEMTKNQVSLTCLVKGFYPSDIAVEWESNGQPENNYKTTPPVLDSDGSFFLYSRLTVDKSRWQEGNVFSCSVMHEALHNHYTQKSLSLSLG